European Patent Application EP 4 589 011 A1, published July 23, 2025. Title: Reagent for tyrosine kinase assay and use thereof. Applicant: ＨＩＬＯ株式会社. The sequence listing filed with the application follows.

SEQUENCE LISTING (7 sequences)

SEQ ID NO: 1 - protein, 303 aa, Homo sapiens
MSSARFDSSDRSAWYMGPVSRQEAQTRLQGQRHGMFLVRDSSTCPGDYVLSVSENSRVSHYIINSLPNRRFKIGDQEFDHLPALLEFYKIHYLDTTTLIEPAPRYPSPPMGSVSAPNLPTAEDNLEYVRTLYDFPGNDAEDLPFKKGEILVIIEKPEEQWWSARNKDGRVGMIPVPYVEKLVRSSPHGKHGNRNSNSYGIPEPAHAYAQPQTTTPLPAVSGSPGAAITPLPSTQNGPVFAKAIQKRVPCAYDKTALALEVGDIVKVTRMNINGQWEGEVNGRKGLFPFTHVKIFDPQNPDENE

SEQ ID NO: 2 - protein, 5 aa, synthetic construct
GGSGG

SEQ ID NO: 3 - protein, 10 aa, Homo sapiens
LALKLAGLDI

SEQ ID NO: 4 - protein, 699 aa, synthetic construct
MVSKGEELFTGVVPILVELDGDVNGHKFSVSGEGEGDATYGKLTLKLICTTGKLPVPWPTLVTTLGYGLQCFARYPDHMKQHDFFKSAMPEGYVQERTIFFKDDGNYKTRAEVKFEGDTLVNRIELKGIDFKEDGNILGHKLEYNYNSHNVYITADKQKNGIKANFKIRHNIEDGGVQLADHYQQNTPIGDGPVLLPDNHYLSYQSALSKDPNEKRDHMVLLEFVTAALEMSSARFDSSDRSAWYMGPVSRQEAQTRLQGQRHGMFLVRDSSTCPGDYVLSVSENSRVSHYIINSLPNRRFKIGDQEFDHLPALLEFYKIHYLDTTTLIEPAPRYPSPPMGSVSAPNLPTAEDNLEYVRTLYDFPGNDAEDLPFKKGEILVIIEKPEEQWWSARNKDGRVGMIPVPYVEKLVRSSPHGKHGNRNSNSYGIPEPAHAYAQPQTTTPLPAVSGSRGRDGSVQLADHYQQNTPIGDGPVLLPDNHYLSTQSALSKDPNEKRDHMVLLEFVTAAGITLGMDELYKGGSGGMVSKGEELFTGVVPILVELDGDVNGHRFSVSGEGEGDATYGKLTLKFICTTGKLPVPWPTLVTTLTWGVQCFSRYPDHMKQHDFFKSAMPEGYVQERTIFFKDDGNYKTRAEVKFEGDTLVNRIELKGIDFKEDGNILGHKLEYNYISHNVYITADKQKNGIKAHFKIRHNIE

SEQ ID NO: 5 - protein, 699 aa, synthetic construct
MVSKGEELFTGVVPILVELDGDVNGHKFSVSGEGEGDATYGKLTLKLICTTGKLPVPWPTLVTTLGYGLQCFARYPDHMKQHDFFKSAMPEGYVQERTIFFKDDGNYKTRAEVKFEGDTLVNRIELKGIDFKEDGNILGHKLEYNYNSHNVYITADKQKNGIKANFKIRHNIEDGGVQLADHYQQNTPIGDGPVLLPDNHYLSYQSKLSKDPNEKRDHMVLLEFVTAALEMSSARFDSSDRSAWYMGPVSRQEAQTRLQGQRHGMFLVRDSSTCPGDYVLSVSENSRVSHYIINSLPNRRFKIGDQEFDHLPALLEFYKIHYLDTTTLIEPAPRYPSPPMGSVSAPNLPTAEDNLEYVRTLYDFPGNDAEDLPFKKGEILVIIEKPEEQWWSARNKDGRVGMIPVPYVEKLVRSSPHGKHGNRNSNSYGIPEPAHAYAQPQTTTPLPAVSGSRGRDGSVQLADHYQQNTPIGDGPVLLPDNHYLSTQSALSKDPNEKRDHMVLLEFVTAAGITLGMDELYKGGSGGMVSKGEELFTGVVPILVELDGDVNGHRFSVSGEGEGDATYGKLTLKFICTTGKLPVPWPTLVTTLTWGVQCFSRYPDHMKQHDFFKSAMPEGYVQERTIFFKDDGNYKTRAEVKFEGDTLVNRIELKGIDFKEDGNILGHKLEYNYISHNVYITADKQKNGIKAHFKIRHNIE

SEQ ID NO: 6 - protein, 699 aa, synthetic construct
MVSKGEELFTGVVPILVELDGDVNGHKFSVSGEGEGDATYGKLTLKLICTTGKLPVPWPTLVTTLGYGLQCFARYPDHMKQHDFFKSAMPEGYVQERTIFFKDDGNYKTRAEVKFEGDTLVNRIELKGIDFKEDGNILGHKLEYNYNSHNVYITADKQKNGIKANFKIRHNIEDGGVQLADHYQQNTPIGDGPVLLPDNHYLSYQSKLSKDPNEKRDHMVLLEFVTAALEMSSARFDSSDRSAWYMGPVSRQEAQTRLQGQRHGMFLVRDSSTCPGDYVLSVSENSRVSHYIINSLPNRRFKIGDQEFDHLPALLEFYKIHYLATTTLIEPAPRYPSPPMGSVSAPNLPTAEDNLEYVRTLYDFPGNDAEDLPFKKGEILVIIEKPEEQWWSARNKDGRVGMIPVPYVEKLVRSSPHGKHGNRNSNSYGIPEPAHAYAQPQTTTPLPAVSGSRGRDGSVQLADHYQQNTPIGDGPVLLPDNHYLSTQSALSKDPNEKRDHMVLLEFVTAAGITLGMDELYKGGSGGMVSKGEELFTGVVPILVELDGDVNGHRFSVSGEGEGDATYGKLTLKFICTTGKLPVPWPTLVTTLTWGVQCFSRYPDHMKQHDFFKSAMPEGYVQERTIFFKDDGNYKTRAEVKFEGDTLVNRIELKGIDFKEDGNILGHKLEYNYISHNVYITADKQKNGIKAHFKIRHNIE

SEQ ID NO: 7 - protein, 715 aa, synthetic construct
MNELALKLAGLDIEFGMVSKGEELFTGVVPILVELDGDVNGHKFSVSGEGEGDATYGKLTLKLICTTGKLPVPWPTLVTTLGYGLQCFARYPDHMKQHDFFKSAMPEGYVQERTIFFKDDGNYKTRAEVKFEGDTLVNRIELKGIDFKEDGNILGHKLEYNYNSHNVYITADKQKNGIKANFKIRHNIEDGGVQLADHYQQNTPIGDGPVLLPDNHYLSYQSKLSKDPNEKRDHMVLLEFVTAALEMSSARFDSSDRSAWYMGPVSRQEAQTRLQGQRHGMFLVRDSSTCPGDYVLSVSENSRVSHYIINSLPNRRFKIGDQEFDHLPALLEFYKIHYLATTTLIEPAPRYPSPPMGSVSAPNLPTAEDNLEYVRTLYDFPGNDAEDLPFKKGEILVIIEKPEEQWWSARNKDGRVGMIPVPYVEKLVRSSPHGKHGNRNSNSYGIPEPAHAYAQPQTTTPLPAVSGSRGRDGSVQLADHYQQNTPIGDGPVLLPDNHYLSTQSALSKDPNEKRDHMVLLEFVTAAGITLGMDELYKGGSGGMVSKGEELFTGVVPILVELDGDVNGHRFSVSGEGEGDATYGKLTLKFICTTGKLPVPWPTLVTTLTWGVQCFSRYPDHMKQHDFFKSAMPEGYVQERTIFFKDDGNYKTRAEVKFEGDTLVNRIELKGIDFKEDGNILGHKLEYNYISHNVYITADKQKNGIKAHFKIRHNIE